European Patent Specification EP 3 837 286 B1, published February 11, 2026. Title: COMPOSITIONS AND METHODS FOR DETECTING AUTOANTIBODIES. Applicant: The Johns Hopkins University. The sequence listing filed with the application follows.

SEQUENCE LISTING (62 sequences)

SEQ ID NO: 1 - DNA, 1404 bp, Artificial Sequence
  mAB12 heavy chain
atggacatgagggtgcccgctcagctcctggggctcctgctgctgtggctgagaggtgcgcgctgtcagatccagttggtgcagtctggacctgagctgaagaagcctggagagacagtcaagatctcctgcaaggcttctgggtataccttcacaaactatccaatgcactgggtgaagcagactccaggaaagggtttaaagtggatgggctggataaacacctactctggagtgccaacatatggagatgacttcaagggacggtttgccttctctttggaaacctctgccagtactgcatatttgcagatcaacaacctcaaaaatgaagacatggctacatatttctgtgcaagatcgaacccctatgattacttgtatgctatggactcctggggtcaaggaacctcagtcaccgtctctagtgccaaaacgacacccccatctgtctacccactggcccctggatctgctgcccaaactaactccatggtgaccctgggatgcctggtcaagggctatttccctgagccagtgacagtgacctggaactctggatccctgtccagcggtgtgcacaccttcccagctgtcctgcagtctgacctctacactctgagcagctcagtgactgtcccctccagcacctggcccagcgagaccgtcacctgcaacgttgcccacccggccagcagcaccaaggtggacaagaaaattgtgcccagggattgtggttgtaagccttgcatatgtacagtcccagaagtatcatctgtcttcatcttccccccaaagcccaaggatgtgctcaccattactctgactcctaaggtcacgtgtgttgtggtagacatcagcaaggatgatcccgaggtccagttcagctggtttgtagatgatgtggaggtgcacacagctcagacgcaaccccgggaggagcagttcaacagcactttccgctcagtcagtgaacttcccatcatgcaccaggactggctcaatggcaaggagttcaaatgcagggtcaacagtgcagctttccctgcccccatcgagaaaaccatctccaaaaccaaaggcagaccgaaggctccacaggtgtacaccattccacctcccaaggagcagatggccaaggataaagtcagtctgacctgcatgataacagacttcttccctgaagacattactgtggagtggcagtggaatgggcagccagcggagaactacaagaacactcagcccatcatggacacagatggctcttacttcgtctacagcaagctcaatgtgcagaagagcaactgggaggcaggaaatactttcacctgctctgtgttacatgagggcctgcacaaccaccatactgagaagagcctctcccactctcctggtaaatga

SEQ ID NO: 2 - protein, 467 aa, Artificial Sequence
  mAB12 heavy chain
MDMRVPAQLLGLLLLWLRGARCQIQLVQSGPELKKPGETVKISCKASGYTFTNYPMHWVKQTPGKGLKWMGWINTYSGVPTYGDDFKGRFAFSLETSASTAYLQINNLKNEDMATYFCARSNPYDYLYAMDSWGQGTSVTVSSAKTTPPSVYPLAPGSAAQTNSMVTLGCLVKGYFPEPVTVTWNSGSLSSGVHTFPAVLQSDLYTLSSSVTVPSSTWPSETVTCNVAHPASSTKVDKKIVPRDCGCKPCICTVPEVSSVFIFPPKPKDVLTITLTPKVTCVVVDISKDDPEVQFSWFVDDVEVHTAQTQPREEQFNSTFRSVSELPIMHQDWLNGKEFKCRVNSAAFPAPIEKTISKTKGRPKAPQVYTIPPPKEQMAKDKVSLTCMITDFFPEDITVEWQWNGQPAENYKNTQPIMDTDGSYFVYSKLNVQKSNWEAGNTFTCSVLHEGLHNHHTEKSLSHSPGK

SEQ ID NO: 3 - protein, 7 aa, Artificial Sequence
  mAb12 heavy chain CDR1
GYTFTNY

SEQ ID NO: 4 - protein, 5 aa, Artificial Sequence
  mAb12 heavy chain CDR2
TYSGV

SEQ ID NO: 5 - protein, 12 aa, Artificial Sequence
  mAB heavy chain CDR3
SNPYDYLYAMDS

SEQ ID NO: 6 - DNA, 726 bp, Artificial Sequence
  mAb12 light chain
atggacatgagggtgcccgctcagctcctggggctcctgctgctgtggctgagaggtgcgcgctgtgatgttgtgatgacccaaactccactctccctgcctgtcagtcttggagatcaagcctccatctcctgcagatctagtcagagccttgtacacatcaatggaaacacctatatacattggtacctgcagaagccaggccagtctccaaagctcctgatctacaaagtttccaaccgattttctggggtcccagacaggttcagtggcagtggatcagggacagattttacactcaagatcagaagagtggaggctgaggatctgggagtttatttctgctctcaaaatacacatgttccattcacattcggctcggggacaaagttggaaataaaacgtgcagatgctgcgccaactgtatccatcttcccaccatctagcgagcagttaacatctggaggtgcctcagtcgtgtgcttcttgaacaacttctaccccaaagacatcaatgtcaagtggaagattgatggcagtgaacgacaaaatggcgtcctgaacagttggactgatcaggacagcaaagacagcacctacagcatgagcagcaccctcacgttgaccaaggacgagtatgaacgacataacagctatacctgtgaggccactcacaagacatcaacttcacccattgtcaagagcttcaacaggaatgagtgttag

SEQ ID NO: 7 - protein, 241 aa, Artificial Sequence
  mAb12 light chain
MDMRVPAQLLGLLLLWLRGARCDVVMTQTPLSLPVSLGDQASISCRSSQSLVHINGNTYIHWYLQKPGQSPKLLIYKVSNRFSGVPDRFSGSGSGTDFTLKIRRVEAEDLGVYFCSQNTHVPFTFGSGTKLEIKRADAAPTVSIFPPSSEQLTSGGASVVCFLNNFYPKDINVKWKIDGSERQNGVLNSWTDQDSKDSTYSMSSTLTLTKDEYERHNSYTCEATHKTSTSPIVKSFNRNEC

SEQ ID NO: 8 - protein, 16 aa, Artificial Sequence
  mAb12 light chain CDR1
RSSQSLVHINGNTYIH

SEQ ID NO: 9 - protein, 7 aa, Artificial Sequence
  mAb12 light chain CDR2
KVSNRFS

SEQ ID NO: 10 - protein, 9 aa, Artificial Sequence
  mAb12 light chain CDR3
SQNTHVPFT

SEQ ID NO: 11 - DNA, 1401 bp, Artificial Sequence
  mAb16 heavy chain
atggacatgagggtgcccgctcagctcctggggctcctgctgctgtggctgagaggtgcgcgctgtcagatccagttggtgcagtctggacctgagctgaagaagcctggagagacagtcacgatctcctgcaaggcttctggatataccttcacacactatccagtgcactgggtgaagcaggctccaggaaagggtttacagtggatgggctggataaacacctactctggagtgccaacatatgcagatgccttcaagaaacgttttgccttctctttggaaacctctgccagcactgcatatttgcagatcaacaacctcaaaagtgaggacatggctacatatttctgtgcaagatcgagggtctatgatgggtactattttgactactggggccaaggcaccactctcaccgtctctagtgccaaaacgacacccccatctgtctacccactggcccctggatctgctgcccaaactaactccatggtgaccctgggatgcctggtcaagggctatttccctgagccagtgacagtgacctggaactctggatccctgtccagcggtgtgcacaccttcccagctgtcctgcagtctgacctctacactctgagcagctcagtgactgtcccctccagcacctggcccagcgagaccgtcacctgcaacgttgcccacccggccagcagcaccaaggtggacaagaaaattgtgcccagggattgtggttgtaagccttgcatatgtacagtcccagaagtatcatctgtcttcatcttccccccaaagcccaaggatgtgctcaccattactctgactcctaaggtcacgtgtgttgtggtagacatcagcaaggatgatcccgaggtccagttcagctggtttgtagatgatgtggaggtgcacacagctcagacgcaaccccgggaggagcagttcaacagcactttccgctcagtcagtgaacttcccatcatgcaccaggactggctcaatggcaaggagttcaaatgcagggtcaacagtgcagctttccctgcccccatcgagaaaaccatctccaaaaccaaaggcagaccgaaggctccacaggtgtacaccattccacctcccaaggagcagatggccaaggataaagtcagtctgacctgcatgataacagacttcttccctgaagacattactgtggagtggcagtggaatgggcagccagcggagaactacaagaacactcagcccatcatggacacagatggctcttacttcgtctacagcaagctcaatgtgcagaagagcaactgggaggcaggaaatactttcacctgctctgtgttacatgagggcctgcacaaccaccatactgagaagagcctctcccactctcctggtaaatga

SEQ ID NO: 12 - protein, 466 aa, Artificial Sequence
  mAb16 heavy chain
MDMRVPAQLLGLLLLWLRGARCQIQLVQSGPELKKPGETVTISCKASGYTFTHYPVHWVKQAPGKGLQWMGWINTYSGVPTYADAFKKRFAFSLETSASTAYLQINNLKSEDMATYFCARSRVYDGYYFDYWGQGTTLTVSSAKTTPPSVYPLAPGSAAQTNSMVTLGCLVKGYFPEPVTVTWNSGSLSSGVHTFPAVLQSDLYTLSSSVTVPSSTWPSETVTCNVAHPASSTKVDKKIVPRDCGCKPCICTVPEVSSVFIFPPKPKDVLTITLTPKVTCVVVDISKDDPEVQFSWFVDDVEVHTAQTQPREEQFNSTFRSVSELPIMHQDWLNGKEFKCRVNSAAFPAPIEKTISKTKGRPKAPQVYTIPPPKEQMAKDKVSLTCMITDFFPEDITVEWQWNGQPAENYKNTQPIMDTDGSYFVYSKLNVQKSNWEAGNTFTCSVLHEGLHNHHTEKSLSHSPGK

SEQ ID NO: 13 - protein, 7 aa, Artificial Sequence
  mAb16 heavy chain CDR1
GYTFTHY

SEQ ID NO: 14 - protein, 6 aa, Artificial Sequence
  mAb16 heavy chain CDR2
NTYSGV

SEQ ID NO: 15 - protein, 11 aa, Artificial Sequence
  mAb16 heavy chain CDR3
SRVYDGYYFDY

SEQ ID NO: 16 - DNA, 726 bp, Artificial Sequence
  mAb16 light chain
atggacatgagggtgcccgctcagctcctggggctcctgctgctgtggctgagaggtgcgcgctgtgatgttgtgatgacccaaactccactctccctgcctgtcagtcttggagatcaagcctccatctcttgcagatctagtcagagccttgtacacagtaatggaaagacctatttacattggtacctgcagaagccaggccagtctccaaacctcctgatctacaaagtttccaaccgattttctggggtcccagacaggttcagtggcagtggatcagggacagatttcacactcaagatcagcagagtggaggctgaggatctgggagtttatttctgctctcaacttacacatgttccgtggacgttcggtggaggcaccaagctggaaatcaaacgtgcagatgctgcgccaactgtatccatcttcccaccatctagcgagcagttaacatctggaggtgcctcagtcgtgtgcttcttgaacaacttctaccccaaagacatcaatgtcaagtggaagattgatggcagtgaacgacaaaatggcgtcctgaacagttggactgatcaggacagcaaagacagcacctacagcatgagcagcaccctcacgttgaccaaggacgagtatgaacgacataacagctatacctgtgaggccactcacaagacatcaacttcacccattgtcaagagcttcaacaggaatgagtgttag

SEQ ID NO: 17 - protein, 241 aa, Artificial Sequence
  mAb16 light chain
MDMRVPAQLLGLLLLWLRGARCDVVMTQTPLSLPVSLGDQASISCRSSQSLVHSNGKTYLHWYLQKPGQSPNLLIYKVSNRFSGVPDRFSGSGSGTDFTLKISRVEAEDLGVYFCSQLTHVPWTFGGGTKLEIKRADAAPTVSIFPPSSEQLTSGGASVVCFLNNFYPKDINVKWKIDGSERQNGVLNSWTDQDSKDSTYSMSSTLTLTKDEYERHNSYTCEATHKTSTSPIVKSFNRNEC

SEQ ID NO: 18 - protein, 16 aa, Artificial Sequence
  mAb16 light chain CDR1
RSSQSLVHSNGKTYLH

SEQ ID NO: 19 - protein, 7 aa, Artificial Sequence
  mAb16 light chain CDR2
KVSNRFS

SEQ ID NO: 20 - protein, 8 aa, Artificial Sequence
  mAb16 light chain CDR3
SQLTHVPW

SEQ ID NO: 21 - DNA, 1407 bp, Artificial Sequence
  mAb17 heavy chain
atggacatgagggtgcccgctcagctcctggggctcctgctgctgtggctgagaggtgcgcgctgtcagatccagttggtgcagtctggacctgagctgaagaagcctggagagacagtcaagatctcctgcaaggcttctgggtataccttcacaaactatccaatgcactggttgaagcaggctccaggaaagggtttaaagtggatgggctggataaacacctactctggagtgccaacatatgcagatgacttcaagggacggtttgccttctctttggaaacctctgccagcactgcatatttgcagatcaacaacctcaaaaatgaggacatggctacatatttctgtacaaaatcgcgcattactacgatggggggttatgctatggactgctggggtcaaggaacctcagtcaccgtctctagtgccaaaacgacacccccatctgtctacccactggcccctggatctgctgcccaaactaactccatggtgaccctgggatgcctggtcaagggctatttccctgagccagtgacagtgacctggaactctggatccctgtccagcggtgtgcacaccttcccagctgtcctgcagtctgacctctacactctgagcagctcagtgactgtcccctccagcacctggcccagcgagaccgtcacctgcaacgttgcccacccggccagcagcaccaaggtggacaagaaaattgtgcccagggattgtggttgtaagccttgcatatgtacagtcccagaagtatcatctgtcttcatcttccccccaaagcccaaggatgtgctcaccattactctgactcctaaggtcacgtgtgttgtggtagacatcagcaaggatgatcccgaggtccagttcagctggtttgtagatgatgtggaggtgcacacagctcagacgcaaccccgggaggagcagttcaacagcactttccgctcagtcagtgaacttcccatcatgcaccaggactggctcaatggcaaggagttcaaatgcagggtcaacagtgcagctttccctgcccccatcgagaaaaccatctccaaaaccaaaggcagaccgaaggctccacaggtgtacaccattccacctcccaaggagcagatggccaaggataaagtcagtctgacctgcatgataacagacttcttccctgaagacattactgtggagtggcagtggaatgggcagccagcggagaactacaagaacactcagcccatcatggacacagatggctcttacttcgtctacagcaagctcaatgtgcagaagagcaactgggaggcaggaaatactttcacctgctctgtgttacatgagggcctgcacaaccaccatactgagaagagcctctcccactctcctggtaaatga

SEQ ID NO: 22 - protein, 468 aa, Artificial Sequence
  mAb17 heavy chain
MDMRVPAQLLGLLLLWLRGARCQIQLVQSGPELKKPGETVKISCKASGYTFTNYPMHWLKQAPGKGLKWMGWINTYSGVPTYADDFKGRFAFSLETSASTAYLQINNLKNEDMATYFCTKSRITTMGGYAMDCWGQGTSVTVSSAKTTPPSVYPLAPGSAAQTNSMVTLGCLVKGYFPEPVTVTWNSGSLSSGVHTFPAVLQSDLYTLSSSVTVPSSTWPSETVTCNVAHPASSTKVDKKIVPRDCGCKPCICTVPEVSSVFIFPPKPKDVLTITLTPKVTCVVVDISKDDPEVQFSWFVDDVEVHTAQTQPREEQFNSTFRSVSELPIMHQDWLNGKEFKCRVNSAAFPAPIEKTISKTKGRPKAPQVYTIPPPKEQMAKDKVSLTCMITDFFPEDITVEWQWNGQPAENYKNTQPIMDTDGSYFVYSKLNVQKSNWEAGNTFTCSVLHEGLHNHHTEKSLSHSPGK

SEQ ID NO: 23 - protein, 7 aa, Artificial Sequence
  mAb17 heavy chain CDR1
GYTFTNY

SEQ ID NO: 24 - protein, 6 aa, Artificial Sequence
  mAb17 heavy chain CDR2
NTYSGV

SEQ ID NO: 25 - protein, 13 aa, Artificial Sequence
  mAb17 heavy chain CDR3
SRITTMGGYAMDC

SEQ ID NO: 26 - DNA, 726 bp, Artificial Sequence
  mAb17 light chain
atggacatgagggtgcccgctcagctcctggggctcctgctgctgtggctgagaggtgcgcgctgtgaagttgtgatgacccaaactccactctccctgcctgtcagtcttggagatcaagcctccatctcttgcagatctagtcagagccttctacacagtaatggaaacacctatttacattggtacctgcagaggccaggccagtctccaaacctcctgatctccaaagtttccaaccgattttctggggtcccagacaggttcagtggcagtggatcagggacagatttcacactcaagatcagcagagtggaggctgaggatctgggagtttatttctgctctcaaaatacacatgttccgtggacgttcggtggaggcaccaagctggaaatcaaacgtgcagatgctgcgccaactgtatccatcttcccaccatctagcgagcagttaacatctggaggtgcctcagtcgtgtgcttcttgaacaacttctaccccaaagacatcaatgtcaagtggaagattgatggcagtgaacgacaaaatggcgtcctgaacagttggactgatcaggacagcaaagacagcacctacagcatgagcagcaccctcacgttgaccaaggacgagtatgaacgacataacagctatacctgtgaggccactcacaagacatcaacttcacccattgtcaagagcttcaacaggaatgagtgttag

SEQ ID NO: 27 - protein, 241 aa, Artificial Sequence
  mAb17 light chain
MDMRVPAQLLGLLLLWLRGARCEVVMTQTPLSLPVSLGDQASISCRSSQSLLHSNGNTYLHWYLQRPGQSPNLLISKVSNRFSGVPDRFSGSGSGTDFTLKISRVEAEDLGVYFCSQNTHVPWTFGGGTKLEIKRADAAPTVSIFPPSSEQLTSGGASVVCFLNNFYPKDINVKWKIDGSERQNGVLNSWTDQDSKDSTYSMSSTLTLTKDEYERHNSYTCEATHKTSTSPIVKSFNRNEC

SEQ ID NO: 28 - protein, 16 aa, Artificial Sequence
  mAb17 light chain CDR1
RSSQSLLHSNGNTYLH

SEQ ID NO: 29 - protein, 7 aa, Artificial Sequence
  mAb17 light chain CDR2
KVSNRFS

SEQ ID NO: 30 - protein, 9 aa, Artificial Sequence
  mAb17 light chain CDR3
SQNTHVPWT

SEQ ID NO: 31 - DNA, 1407 bp, Artificial Sequence
  mAb20 heavy chain
atggacatgagggtgcccgctcagctcctggggctcctgctgctgtggctgagaggtgcgcgctgtcagatccagttggtgcagtctggacctgagctgaagaagcctggagagacagtcaagatctcctgcaaggcttctgggtatatcttcacaaactatccaatgcactgggtgaagcaggctccaggaaagggtttaaagtggatgggctggataaacacctactctggagtgccaacacatgcagatgacttcaagggacggtttgccttctctttggaaacctctgccaacagtgcatttttgcagatcaacaacctcaaaaatgaggacacggctacatatttctgtacaagatcgcgcattactccgacggggggctatgctatggactactggggtcaaggaacctcagtcaccgtctctagtgccaaaacgacacccccatctgtctacccactggcccctggatctgctgcccaaactaactccatggtgaccctgggatgcctggtcaagggctatttccctgagccagtgacagtgacctggaactctggatccctgtccagcggtgtgcacaccttcccagctgtcctgcagtctgacctctacactctgagcagctcagtgactgtcccctccagcacctggcccagcgagaccgtcacctgcaacgttgcccacccggccagcagcaccaaggtggacaagaaaattgtgcccagggattgtggttgtaagccttgcatatgtacagtcccagaagtatcatctgtcttcatcttccccccaaagcccaaggatgtgctcaccattactctgactcctaaggtcacgtgtgttgtggtagacatcagcaaggatgatcccgaggtccagttcagctggtttgtagatgatgtggaggtgcacacagctcagacgcaaccccgggaggagcagttcaacagcactttccgctcagtcagtgaacttcccatcatgcaccaggactggctcaatggcaaggagttcaaatgcagggtcaacagtgcagctttccctgcccccatcgagaaaaccatctccaaaaccaaaggcagaccgaaggctccacaggtgtacaccattccacctcccaaggagcagatggccaaggataaagtcagtctgacctgcatgataacagacttcttccctgaagacattactgtggagtggcagtggaatgggcagccagcggagaactacaagaacactcagcccatcatggacacagatggctcttacttcgtctacagcaagctcaatgtgcagaagagcaactgggaggcaggaaatactttcacctgctctgtgttacatgagggcctgcacaaccaccatactgagaagagcctctcccactctcctggtaaatga

SEQ ID NO: 32 - protein, 468 aa, Artificial Sequence
  mAb20 heavy chain
MDMRVPAQLLGLLLLWLRGARCQIQLVQSGPELKKPGETVKISCKASGYIFTNYPMHWVKQAPGKGLKWMGWINTYSGVPTHADDFKGRFAFSLETSANSAFLQINNLKNEDTATYFCTRSRITPTGGYAMDYWGQGTSVTVSSAKTTPPSVYPLAPGSAAQTNSMVTLGCLVKGYFPEPVTVTWNSGSLSSGVHTFPAVLQSDLYTLSSSVTVPSSTWPSETVTCNVAHPASSTKVDKKIVPRDCGCKPCICTVPEVSSVFIFPPKPKDVLTITLTPKVTCVVVDISKDDPEVQFSWFVDDVEVHTAQTQPREEQFNSTFRSVSELPIMHQDWLNGKEFKCRVNSAAFPAPIEKTISKTKGRPKAPQVYTIPPPKEQMAKDKVSLTCMITDFFPEDITVEWQWNGQPAENYKNTQPIMDTDGSYFVYSKLNVQKSNWEAGNTFTCSVLHEGLHNHHTEKSLSHSPGK

SEQ ID NO: 33 - protein, 7 aa, Artificial Sequence
  mAb20 heavy chain CDR1
GYIFTNY

SEQ ID NO: 34 - protein, 6 aa, Artificial Sequence
  mAb20 heavy chain CDR2
NTYSGV

SEQ ID NO: 35 - protein, 13 aa, Artificial Sequence
  mAb20 heavy chain CDR3
SRITPTGGYAMDY

SEQ ID NO: 36 - DNA, 726 bp, Artificial Sequence
  mAb20 light chain
atggacatgagggtgcccgctcagctcctggggctcctgctgctgtggctgagaggtgcgcgctgtgatgttgtgatgacccaaactccactctccctgcctgtcagtcttggagatcaagcctccatctcttgcagatctagtcagagccttgtacacagtaatggaaacacctatttacattggtacctgcagaagccaggccagtctccaaacctcctgatctccaaagtttccaaccgattttctggggtcccagaaaggttcagtggcagtggatcagggacagatttcacactcaagatcagcagagtggaggctgaggatctgggagtttatttctgctctcaaaatacacatgttccgtggacgttcggtggaggcaccaagctggaaatcaaacgtgcagatgctgcgccaactgtatccatcttcccaccatctagcgagcagttaacatctggaggtgcctcagtcgtgtgcttcttgaacaacttctaccccaaagacatcaatgtcaagtggaagattgatggcagtgaacgacaaaatggcgtcctgaacagttggactgatcaggacagcaaagacagcacctacagcatgagcagcaccctcacgttgaccaaggacgagtatgaacgacataacagctatacctgtgaggccactcacaagacatcaacttcacccattgtcaagagcttcaacaggaatgagtgttag

SEQ ID NO: 37 - protein, 241 aa, Artificial Sequence
  mAb20 light chain
MDMRVPAQLLGLLLLWLRGARCDVVMTQTPLSLPVSLGDQASISCRSSQSLVHSNGNTYLHWYLQKPGQSPNLLISKVSNRFSGVPERFSGSGSGTDFTLKISRVEAEDLGVYFCSQNTHVPWTFGGGTKLEIKRADAAPTVSIFPPSSEQLTSGGASVVCFLNNFYPKDINVKWKIDGSERQNGVLNSWTDQDSKDSTYSMSSTLTLTKDEYERHNSYTCEATHKTSTSPIVKSFNRNEC

SEQ ID NO: 38 - protein, 16 aa, Artificial Sequence
  mAb20 light chain CDR1
RSSQSLVHSNGNTYLH

SEQ ID NO: 39 - protein, 7 aa, Artificial Sequence
  mAb20 light chain CDR2
KVSNRFS

SEQ ID NO: 40 - protein, 9 aa, Artificial Sequence
  mAb40 light chain CDR3
SQNTHVPWT

SEQ ID NO: 41 - DNA, 1407 bp, Artificial Sequence
  mAb28 heavy chain
atggacatgagggtgcccgctcagctcctggggctcctgctgctgtggctgagaggtgcgcgctgtcagatccagttggtgcagtctggacctgagctgaagaagcctggagagacagtcaagatctcctgcaaggcttctgggtataccttcacaaactatccaatgcactgggtaaagcaggctccaggaaaggatttaaagtggatgggctggataaacacctactctggaatgtcaacatatgcagatgacttcaagggacggtttgccttctctttggaaacctctgccagcactgcgtatttgcagatcaacaacctcaaaaatgaggacatggctacatatttctgtgcaagatcgcgcattacaacgatggggggctatgctatggactactggggtcaaggagcctcagtcaccgtctctagtgccaaaacgacacccccatctgtctacccactggcccctggatctgctgcccaaactaactccatggtgaccctgggatgcctggtcaagggctatttccctgagccagtgacagtgacctggaactctggatccctgtccagcggtgtgcacaccttcccagctgtcctgcagtctgacctctacactctgagcagctcagtgactgtcccctccagcacctggcccagcgagaccgtcacctgcaacgttgcccacccggccagcagcaccaaggtggacaagaaaattgtgcccagggattgtggttgtaagccttgcatatgtacagtcccagaagtatcatctgtcttcatcttccccccaaagcccaaggatgtgctcaccattactctgactcctaaggtcacgtgtgttgtggtagacatcagcaaggatgatcccgaggtccagttcagctggtttgtagatgatgtggaggtgcacacagctcagacgcaaccccgggaggagcagttcaacagcactttccgctcagtcagtgaacttcccatcatgcaccaggactggctcaatggcaaggagttcaaatgcagggtcaacagtgcagctttccctgcccccatcgagaaaaccatctccaaaaccaaaggcagaccgaaggctccacaggtgtacaccattccacctcccaaggagcagatggccaaggataaagtcagtctgacctgcatgataacagacttcttccctgaagacattactgtggagtggcagtggaatgggcagccagcggagaactacaagaacactcagcccatcatggacacagatggctcttacttcgtctacagcaagctcaatgtgcagaagagcaactgggaggcaggaaatactttcacctgctctgtgttacatgagggcctgcacaaccaccatactgagaagagcctctcccactctcctggtaaatga

SEQ ID NO: 42 - protein, 468 aa, Artificial Sequence
  mAb28 heavy chain
MDMRVPAQLLGLLLLWLRGARCQIQLVQSGPELKKPGETVKISCKASGYTFTNYPMHWVKQAPGKDLKWMGWINTYSGMSTYADDFKGRFAFSLETSASTAYLQINNLKNEDMATYFCARSRITTMGGYAMDYWGQGASVTVSSAKTTPPSVYPLAPGSAAQTNSMVTLGCLVKGYFPEPVTVTWNSGSLSSGVHTFPAVLQSDLYTLSSSVTVPSSTWPSETVTCNVAHPASSTKVDKKIVPRDCGCKPCICTVPEVSSVFIFPPKPKDVLTITLTPKVTCVVVDISKDDPEVQFSWFVDDVEVHTAQTQPREEQFNSTFRSVSELPIMHQDWLNGKEFKCRVNSAAFPAPIEKTISKTKGRPKAPQVYTIPPPKEQMAKDKVSLTCMITDFFPEDITVEWQWNGQPAENYKNTQPIMDTDGSYFVYSKLNVQKSNWEAGNTFTCSVLHEGLHNHHTEKSLSHSPGK

SEQ ID NO: 43 - protein, 7 aa, Artificial Sequence
  mAb28 heavy chain CDR1
GYTFTNY

SEQ ID NO: 44 - protein, 6 aa, Artificial Sequence
  mAb28 heavy chain CDR2
NTYSGM

SEQ ID NO: 45 - protein, 13 aa, Artificial Sequence
  mAb28 heavy chain CDR3
SRITTMGGYAMDY

SEQ ID NO: 46 - DNA, 726 bp, Artificial Sequence
  mAb28 light chain
atggacatgagggtgcccgctcagctcctggggctcctgctgctgtggctgagaggtgcgcgctgtgaagttgtgatgacccaaactccactctccctgcctgtcagtcttggagatcaagcctccatctcttgcagatctagtcagagccttgtacacagtaatggaaacacctatttacattggtacctgcagaagccaggccagtctccaaagctcctgatctccaaagtttccaaccgattttctggggtcccagacaggttcagtggcagtggatcagggacagatttcacactcaagatcatcagagtggaggctgaggatctgggagtttatttctgctctcaaaatacacatgttccgtggacgttcggtggaggcaccaagctggaaatcaaacgtgcagatgctgcgccaactgtatccatcttcccaccatctagcgagcagttaacatctggaggtgcctcagtcgtgtgcttcttgaacaacttctaccccaaagacatcaatgtcaagtggaagattgatggcagtgaacgacaaaatggcgtcctgaacagttggactgatcaggacagcaaagacagcacctacagcatgagcagcaccctcacgttgaccaaggacgagtatgaacgacataacagctatacctgtgaggccactcacaagacatcaacttcacccattgtcaagagcttcaacaggaatgagtgttag

SEQ ID NO: 47 - protein, 241 aa, Artificial Sequence
  mAb28 light chain
MDMRVPAQLLGLLLLWLRGARCEVVMTQTPLSLPVSLGDQASISCRSSQSLVHSNGNTYLHWYLQKPGQSPKLLISKVSNRFSGVPDRFSGSGSGTDFTLKIIRVEAEDLGVYFCSQNTHVPWTFGGGTKLEIKRADAAPTVSIFPPSSEQLTSGGASVVCFLNNFYPKDINVKWKIDGSERQNGVLNSWTDQDSKDSTYSMSSTLTLTKDEYERHNSYTCEATHKTSTSPIVKSFNRNEC

SEQ ID NO: 48 - protein, 16 aa, Artificial Sequence
  mAb28 light chain CDR1
RSSQSLVHSNGNTYLH

SEQ ID NO: 49 - protein, 7 aa, Artificial Sequence
  mAb28 light chain CDR2
KVSNRFS

SEQ ID NO: 50 - protein, 9 aa, Artificial Sequence
  mAb28 light chain CDR3
SQNTHVPWT

SEQ ID NO: 51 - DNA, 1389 bp, Artificial Sequence
  mAb39 heavy chain
atgggatggagctgtatcatgttctttttggtagcaacagctacagatgtccactcccaggtccaactgcagcagcctggggctgaactggtgaagcctggggcttcagtgaagctgtcctgcaaggcttctggctactccttcaccacctactggatgcactgggtgaagcagaggcctggacaaggcctagagtgggttggagatattaatcctaggaacggtcgtactaactacaatgagaagtccaagagcaaggccacactgactgtagacatatcatccagcacagtatacatgcaagtcagcagcctgacatctgaggactctgcggtctattactgtgcaatatggtcgggtgctatggactactggggtccaggaacctcagtcaccgtctcctcagccaaaacaacagccccatcggtctatccactggcccctgtgtgtggagatacaactggctcctcggtgactctaggatgcctggtcaagggttatttccctgagccagtgaccttgacctggaactctggatccctgtccagtgatgtgcacaccttcccagctctcctgcagtctggcctctacaccctcagcagctcagtgactgtaaccacctggcccagccagaccatcacctgcaatgtggcccacccggcaagcagcaccaaagtggacaagaaaattgagcccagagggtccccaacacataaaccctgtcctccatgcccagctcctaacctcttgggtggaccatccgtcttcatcttccctccaaagatcaaggatgtactcatgatctccctgagccccatggtcacgtgtgtggtggtggatgtgagcgaggatgacccagatgtccatgtcagctggttcgtgaacaacgtggaagtacacacagctcagacacaaacccatagagaggattacaacagtactatccgggtggtcagtgccctccccatccagcaccaggactggatgagtggcaaggagttcaaatgcaaggtcaacaacaaagccctcccagcgcccatcgagagaaccatctcaaaacccaaagggccagtaagagctccacaggtatatgtcttgcctccaccagaagaagagatgactaagaaacaggtcactctgacctgcatgatcacagacttcatgcctgaagacatttacgtggagtggaccaacaacgggcaaacagagctaaactacaagaacactgaaccagtcctggactctgatggttcttacttcatgtacagcaagctgagagtggaaaagaagaactgggtggaaagaaatagctactcctgttcagtggtccacgagggtctgcacaatcaccacacgactaagagcttctcccggtctccgggtaaatga

SEQ ID NO: 52 - protein, 462 aa, Artificial Sequence
  mAb39 heavy chain
MGWSCIMFFLVATATDVHSQVQLQQPGAELVKPGASVKLSCKASGYSFTTYWMHWVKQRPGQGLEWVGDINPRNGRTNYNEKSKSKATLTVDISSSTVYMQVSSLTSEDSAVYYCAIWSGAMDYWGPGTSVTVSSAKTTAPSVYPLAPVCGDTTGSSVTLGCLVKGYFPEPVTLTWNSGSLSSDVHTFPALLQSGLYTLSSSVTVTTWPSQTITCNVAHPASSTKVDKKIEPRGSPTHKPCPPCPAPNLLGGPSVFIFPPKIKDVLMISLSPMVTCVVVDVSEDDPDVHVSWFVNNVEVHTAQTQTHREDYNSTIRVVSALPIQHQDWMSGKEFKCKVNNKALPAPIERTISKPKGPVRAPQVYVLPPPEEEMTKKQVTLTCMITDFMPEDIYVEWTNNGQTELNYKNTEPVLDSDGSYFMYSKLRVEKKNWVERNSYSCSVVHEGLHNHHTTKSFSRSPGK

SEQ ID NO: 53 - protein, 7 aa, Artificial Sequence
  mAb39 heavy chain CDR1
GYSFTTY

SEQ ID NO: 54 - protein, 6 aa, Artificial Sequence
  mAb39 heavy chain CDR2
NPRNGR

SEQ ID NO: 55 - protein, 7 aa, Artificial Sequence
  mAb39 heavy chain CDR3
WSGAMDY

SEQ ID NO: 56 - DNA, 717 bp, Artificial Sequence
  mAb39 light chain
atgaagttgcctgttaggctgttggtgctgatgttctggattcctgcttccagcagtgatgttgtgatgacccaaactccactctccctgcctgtcagtcttggagatcaaccctccatctcttgcaaatctagtcagagccttgtacacaataatggaaacacctatttacattggtacctgcagaagccaggccagtctccaaagctcctgatctacaaagtttccaaccgattttctggggtcccagacaggttcagtggcagtggatcagggacagatttcacactcaagatcagcagagtggaggctgaggatctgggagtttatttctgctctcaaactacacatgttcctccgacgttcggtggaggcaccaagctggaaatcaaacgggctgatgctgcaccaactgtatccatcttcccaccatccagtgagcagttaacatctggaggtgcctcagtcgtgtgcttcttgaacaacttctaccccaaagacatcaatgtcaagtggaagattgatggcagtgaacgacaaaatggcgtcctgaacagttggactgatcaggacagcaaagacagcacctacagcatgagcagcaccctcacgttgaccaaggacgagtatgaacgacataacagctatacctgtgaggccactcacaagacatcaacttcacccattgtcaagagcttcaacaggggagagtgttga

SEQ ID NO: 57 - protein, 238 aa, Artificial Sequence
  mAb39 light chain
MKLPVRLLVLMFWIPASSSDVVMTQTPLSLPVSLGDQPSISCKSSQSLVHNNGNTYLHWYLQKPGQSPKLLIYKVSNRFSGVPDRFSGSGSGTDFTLKISRVEAEDLGVYFCSQTTHVPPTFGGGTKLEIKRADAAPTVSIFPPSSEQLTSGGASVVCFLNNFYPKDINVKWKIDGSERQNGVLNSWTDQDSKDSTYSMSSTLTLTKDEYERHNSYTCEATHKTSTSPIVKSFNRGEC

SEQ ID NO: 58 - protein, 16 aa, Artificial Sequence
  mAb39 light chain CDR1
KSSQSLVHNNGNTYLH

SEQ ID NO: 59 - protein, 7 aa, Artificial Sequence
  mAb39 light chain CDR2
KVSNRFS

SEQ ID NO: 60 - protein, 9 aa, Artificial Sequence
  mAb39 light chain CDR3
SQTTHVPPT

SEQ ID NO: 61 - DNA, 1389 bp, Artificial Sequence
  mAb39 heavy chain v2 (t1375a-->S459T)
atgggatggagctgtatcatgttctttttggtagcaacagctacagatgtccactcccaggtccaactgcagcagcctggggctgaactggtgaagcctggggcttcagtgaagctgtcctgcaaggcttctggctactccttcaccacctactggatgcactgggtgaagcagaggcctggacaaggcctagagtgggttggagatattaatcctaggaacggtcgtactaactacaatgagaagtccaagagcaaggccacactgactgtagacatatcatccagcacagtatacatgcaagtcagcagcctgacatctgaggactctgcggtctattactgtgcaatatggtcgggtgctatggactactggggtccaggaacctcagtcaccgtctcctcagccaaaacaacagccccatcggtctatccactggcccctgtgtgtggagatacaactggctcctcggtgactctaggatgcctggtcaagggttatttccctgagccagtgaccttgacctggaactctggatccctgtccagtgatgtgcacaccttcccagctctcctgcagtctggcctctacaccctcagcagctcagtgactgtaaccacctggcccagccagaccatcacctgcaatgtggcccacccggcaagcagcaccaaagtggacaagaaaattgagcccagagggtccccaacacataaaccctgtcctccatgcccagctcctaacctcttgggtggaccatccgtcttcatcttccctccaaagatcaaggatgtactcatgatctccctgagccccatggtcacgtgtgtggtggtggatgtgagcgaggatgacccagatgtccatgtcagctggttcgtgaacaacgtggaagtacacacagctcagacacaaacccatagagaggattacaacagtactatccgggtggtcagtgccctccccatccagcaccaggactggatgagtggcaaggagttcaaatgcaaggtcaacaacaaagccctcccagcgcccatcgagagaaccatctcaaaacccaaagggccagtaagagctccacaggtatatgtcttgcctccaccagaagaagagatgactaagaaacaggtcactctgacctgcatgatcacagacttcatgcctgaagacatttacgtggagtggaccaacaacgggcaaacagagctaaactacaagaacactgaaccagtcctggactctgatggttcttacttcatgtacagcaagctgagagtggaaaagaagaactgggtggaaagaaatagctactcctgttcagtggtccacgagggtctgcacaatcaccacacgactaagagcttctcccggactccgggtaaatga

SEQ ID NO: 62 - protein, 462 aa, Artificial Sequence
  mAb39 heavy chain (S459T)
MGWSCIMFFLVATATDVHSQVQLQQPGAELVKPGASVKLSCKASGYSFTTYWMHWVKQRPGQGLEWVGDINPRNGRTNYNEKSKSKATLTVDISSSTVYMQVSSLTSEDSAVYYCAIWSGAMDYWGPGTSVTVSSAKTTAPSVYPLAPVCGDTTGSSVTLGCLVKGYFPEPVTLTWNSGSLSSDVHTFPALLQSGLYTLSSSVTVTTWPSQTITCNVAHPASSTKVDKKIEPRGSPTHKPCPPCPAPNLLGGPSVFIFPPKIKDVLMISLSPMVTCVVVDVSEDDPDVHVSWFVNNVEVHTAQTQTHREDYNSTIRVVSALPIQHQDWMSGKEFKCKVNNKALPAPIERTISKPKGPVRAPQVYVLPPPEEEMTKKQVTLTCMITDFMPEDIYVEWTNNGQTELNYKNTEPVLDSDGSYFMYSKLRVEKKNWVERNSYSCSVVHEGLHNHHTTKSFSRTPGK